European Patent Application EP 4 534 557 A1, published April 9, 2025. Title: ANTI-BDCA2 ANTIBODY AND USE THEREOF. Applicant: DUALITY BIOLOGICS (SUZHOU) CO., LTD. Application WO. The sequence listing filed with the application follows.

SEQUENCE LISTING (196 sequences)

SEQ ID NO: 1 - protein, 5 aa, synthetic construct
DFSMH

SEQ ID NO: 2 - protein, 17 aa, synthetic construct
WINTETGEPTYADDFKG

SEQ ID NO: 3 - protein, 12 aa, synthetic construct
GGDGHPYWYFAV

SEQ ID NO: 4 - protein, 15 aa, synthetic construct
RASQSVSTSSYSYMH

SEQ ID NO: 5 - protein, 7 aa, synthetic construct
YASILES

SEQ ID NO: 6 - protein, 9 aa, synthetic construct
QHSWEIPFT

SEQ ID NO: 7 - protein, 5 aa, synthetic construct
DYSMH

SEQ ID NO: 8 - protein, 12 aa, synthetic construct
GGDGFPYWYFNV

SEQ ID NO: 9 - protein, 15 aa, synthetic construct
RASQSVSTSSNSYIH

SEQ ID NO: 10 - protein, 7 aa, synthetic construct
YASNLDS

SEQ ID NO: 11 - protein, 5 aa, synthetic construct
NYGVH

SEQ ID NO: 12 - protein, 16 aa, synthetic construct
VIWSGESTDYDAAFIS

SEQ ID NO: 13 - protein, 12 aa, synthetic construct
RRSHYYGYVMDY

SEQ ID NO: 14 - protein, 15 aa, synthetic construct
KASQSIDYDGIGYLN

SEQ ID NO: 15 - protein, 7 aa, synthetic construct
AASNLES

SEQ ID NO: 16 - protein, 9 aa, synthetic construct
QQSNEDPPT

SEQ ID NO: 17 - protein, 5 aa, synthetic construct
SYGVH

SEQ ID NO: 18 - protein, 15 aa, synthetic construct
KASQSVDYDGVGYLN

SEQ ID NO: 19 - protein, 5 aa, synthetic construct
DYYMY

SEQ ID NO: 20 - protein, 17 aa, synthetic construct
YISYSGDSTYYPDTVKG

SEQ ID NO: 21 - protein, 11 aa, synthetic construct
HSPSFPYYFDY

SEQ ID NO: 22 - protein, 10 aa, synthetic construct
SASSSVSYMH

SEQ ID NO: 23 - protein, 7 aa, synthetic construct
EISKLAS

SEQ ID NO: 24 - protein, 9 aa, synthetic construct
QLWNYPLIT

SEQ ID NO: 25 - protein, 6 aa, synthetic construct
SGYYWN

SEQ ID NO: 26 - protein, 16 aa, synthetic construct
YISFDGTYNYNPSLKD

SEQ ID NO: 27 - protein, 10 aa, synthetic construct
GVDYPNAIDW

SEQ ID NO: 28 - protein, 15 aa, synthetic construct
RASESVSMHVTHLIH

SEQ ID NO: 29 - protein, 7 aa, synthetic construct
VASNLES

SEQ ID NO: 30 - protein, 9 aa, synthetic construct
QQSFEDPWT

SEQ ID NO: 31 - protein, 6 aa, synthetic construct
SAYYWN

SEQ ID NO: 32 - protein, 16 aa, synthetic construct
YITYDGNNYYSPSLKN

SEQ ID NO: 33 - protein, 11 aa, synthetic construct
GGDYDDGGFAF

SEQ ID NO: 34 - protein, 11 aa, synthetic construct
RASGNIHNYLA

SEQ ID NO: 35 - protein, 7 aa, synthetic construct
NAKSLVD

SEQ ID NO: 36 - protein, 9 aa, synthetic construct
QHFWIVPYT

SEQ ID NO: 37 - protein, 10 aa, synthetic construct
GVDYPKAMDW

SEQ ID NO: 38 - protein, 5 aa, synthetic construct
SFGMS

SEQ ID NO: 39 - protein, 15 aa, synthetic construct
TISSGDSYTYYPDSV

SEQ ID NO: 40 - protein, 12 aa, synthetic construct
QIYYDYAYYFDY

SEQ ID NO: 41 - protein, 15 aa, synthetic construct
RASESVSFRSSHLMH

SEQ ID NO: 42 - protein, 9 aa, synthetic construct
QQSIEDPPT

SEQ ID NO: 43 - protein, 16 aa, synthetic construct
YISYDGSNNYNPSLKN

SEQ ID NO: 44 - protein, 15 aa, synthetic construct
RASESVSIHGTHLMH

SEQ ID NO: 45 - protein, 7 aa, synthetic construct
VASYLES

SEQ ID NO: 46 - protein, 16 aa, synthetic construct
YITYDGSNNYNPSLKN

SEQ ID NO: 47 - protein, 11 aa, synthetic construct
GGDYDDGGFAY

SEQ ID NO: 48 - protein, 7 aa, synthetic construct
NAKTLVD

SEQ ID NO: 49 - protein, 9 aa, synthetic construct
QHFWIIPYT

SEQ ID NO: 50 - protein, 16 aa, synthetic construct
YISYDGSNYYNPSLKN

SEQ ID NO: 51 - protein, 7 aa, synthetic construct
NAKTLAD

SEQ ID NO: 52 - protein, 5 aa, synthetic construct
SYGMS

SEQ ID NO: 53 - protein, 12 aa, synthetic construct
QIYYDYAYYFDF

SEQ ID NO: 54 - protein, 15 aa, synthetic construct
RASESVSFRTSHLMH

SEQ ID NO: 55 - protein, 7 aa, synthetic construct
GASNLES

SEQ ID NO: 56 - protein, 16 aa, synthetic construct
YITYDGSNNYNPSLKD

SEQ ID NO: 57 - protein, 121 aa, synthetic construct
QIQLVQSGPELKKPGETVKISCKASGYTFTDFSMHWVKQAPGKGLKWMGWINTETGEPTYADDFKGRFAFSLETSASTAFLQINNLKNDDTTTYFCSRGGDGHPYWYFAVWGAGTTVTVSS

SEQ ID NO: 58 - protein, 111 aa, synthetic construct
DIVLTQSPASLAVSLGQRATISCRASQSVSTSSYSYMHWYQQKPGQPPKLLIKYASILESGVPARFSGSGSGTDFTLNIHPVEEEDTATYYCQHSWEIPFTFGSGTKLEIK

SEQ ID NO: 59 - protein, 121 aa, synthetic construct
QIQLVQSGPELKKPGETVKISCRASGYSFTDYSMHWVKQAPGKGLKWVGWINTETGEPTYADDFKGRFALSLETSATSAYLQINNLKNEDTATYFCARGGDGFPYWYFNVWGAGTTVTVSS

SEQ ID NO: 60 - protein, 111 aa, synthetic construct
DIVLTQSPTSLAVSLGQRTNISCRASQSVSTSSNSYIHWYQQKPGQPPKLLIKYASNLDSGVPARFSGSGSGTDFTLNIHPVEEEDTSTYYCQHSWEIPFTFGSGTKLEIK

SEQ ID NO: 61 - protein, 120 aa, synthetic construct
QVQLKQSGPGLVQPSQSLSITCTVSGFSLTNYGVHWVRQSPGKGLEWLGVIWSGESTDYDAAFISRLSISKDNSKSQVFFKMNSLQADDSAIYYCARRRSHYYGYVMDYWGQGTSVTVSS

SEQ ID NO: 62 - protein, 111 aa, synthetic construct
DIVLTQSPASLAVSLGQRATISCKASQSIDYDGIGYLNWYQHKPGQPPKLLIYAASNLESGIPARFSGSGSGTDFTLNIHPVEEEDAATYYCQQSNEDPPTFGSGTKLEIK

SEQ ID NO: 63 - protein, 120 aa, synthetic construct
QVQLKQSGPGLVQPSQSLSITCTVSGFSLTSYGVHWVRQSPGKGLEWLGVIWSGESTDYDAAFISRLSISKDNSKSQVFFRMNSLQADDSAIYYCARRRSHYYGYVMDYWGQGTSVTVSS

SEQ ID NO: 64 - protein, 111 aa, synthetic construct
DIVLTQSPASLAVSLGQRATISCKASQSVDYDGVGYLNWYQHKPGQPPKLLIYAASNLESGIPARFSGSGSGTDFTLNIHPVEEEDAATYYCQQSNEDPPTFGSGTKLEIK

SEQ ID NO: 65 - protein, 120 aa, synthetic construct
EVKLVESGGDLVQPGGSLKLSCAASGFTFSDYYMYWVRQTPEKRLEWVAYISYSGDSTYYPDTVKGRFTISRDNAKNTLFLQMSRLKSEDTAMYYCARHSPSFPYYFDYWGQGTALTVSS

SEQ ID NO: 66 - protein, 106 aa, synthetic construct
EIVLTQSPAITAASLGQKVTITCSASSSVSYMHWYQQKSGTSPKPWIYEISKLASGVPARFSGSGSGTSYSLTISSMEAEDAAIYYCQLWNYPLITFGGGTNLEIK

SEQ ID NO: 67 - protein, 119 aa, synthetic construct
DVQLQESGPGLVKPSQSLSLTCSVTGYSIASGYYWNWIRQFPGNKLEWMGYISFDGTYNYNPSLKDRFSITRDTSKNQFFLKLNSVTTEDTATYYCARGVDYPNAIDWWGQGTSVTVSS

SEQ ID NO: 68 - protein, 111 aa, synthetic construct
DIVLTQSPASLAVSLGQRATISCRASESVSMHVTHLIHWYQQKPGQPPKLLIYVASNLESGVPARFSGSGSETDFTLNIHPVEEEDAATYFCQQSFEDPWTFGGGTKLEIK

SEQ ID NO: 69 - protein, 120 aa, synthetic construct
DVQLQESGPGLVKPSQSLSLTCSVTGYSITSAYYWNWIRQFPGNKLECMGYITYDGNNYYSPSLKNRISITRDTSKNQFFLNLNSVTTEDTATYFCARGGDYDDGGFAFWGQGTLVTVSA

SEQ ID NO: 70 - protein, 107 aa, synthetic construct
DIQMTQSPASLSASVGETVTITCRASGNIHNYLAWYHQKQGKSPQLLVYNAKSLVDGVPSRFSGSGSGTQYSLRINSLQPEDFGSYYCQHFWIVPYTFGGGTKLEII

SEQ ID NO: 71 - protein, 119 aa, synthetic construct
DVQLQESGPGLVKPSQSLSLTCSVTGYSITSGYYWNWIRQFPGNKLEWMGYISFDGTYNYNPSLKDRFSITRDTSKNQFFLKLNSVTTEDTATYYCARGVDYPKAMDWWGQGTSVTVSS

SEQ ID NO: 72 - protein, 121 aa, synthetic construct
EVQLVESGGDLVKPGGSLKLSCAASGFTFSSFGMSWVRQTPDKRLDWVATISSGDSYTYYPDSVKGRFSISRDNAKNTLYLQMSSLKSEDTAVYYCARQIYYDYAYYFDYWGQGTTLTVSS

SEQ ID NO: 73 - protein, 111 aa, synthetic construct
DIVLTQSPASLAVSLGQRATISCRASESVSFRSSHLMHWYRQKPGQPPKLLIYAASNLESGVPARFSGSGSETDFTLNIHPVEEEDAAAYFCQQSIEDPPTFGGGTKLEIK

SEQ ID NO: 74 - protein, 119 aa, synthetic construct
DVQLQESGPGLVKPSQSLSLTCSVTGYSITSAYYWNWIRQFPGHKLEWMGYISYDGSNNYNPSLKNRISITRDTSKNQFFLKLNSVTTEDTATYHCARGVDYPNAIDWWGQGTSLTVSS

SEQ ID NO: 75 - protein, 111 aa, synthetic construct
DIVLTQSPTSLTVSLGQRATISCRASESVSIHGTHLMHWYQQKPGQPPKLLIYVASYLESGVPARFSGSGSETDFSLNIHPVEEEDAATYFCQQSFEDPWTFGGGTKLEIK

SEQ ID NO: 76 - protein, 120 aa, synthetic construct
DVQLQESGPGLVKPSQSLSLTCSVTGYSITSAYYWNWVRQFPGNQLECMGYITYDGSNNYNPSLKNRISITRDTSKNQFFLKLNSVTTEDTATYYCVRGGDYDDGGFAYWGQGTLVTVSA

SEQ ID NO: 77 - protein, 107 aa, synthetic construct
DIQMTQSPASLSASVGETVTITCRASGNIHNYLAWYQQKQGKSPQLLVYNAKTLVDGVPSRFSGSGSGTEYSLKINSLQPEDFGIYFCQHFWIIPYTFGGGTKLEIR

SEQ ID NO: 78 - protein, 120 aa, synthetic construct
DVQLQESGPGLVKPSQSLSLTCSVTGYSISSGYYWNWIRQFPGNKLECMGYISYDGSNYYNPSLKNRISITRDTSKNQFFLSLNSVTTEDTATYFCVRGGDYDDGGFAYWGQGTLVTVSA

SEQ ID NO: 79 - protein, 107 aa, synthetic construct
DIQMTQSPASLSASVGETVTITCRASGNIHNYLAWYQQKQGKSPQLLVYNAKTLADGVPSRFSGSGSETQYSLKINSLQPEDFGNYFCQHFWIIPYTFGGGTKLEIK

SEQ ID NO: 80 - protein, 120 aa, synthetic construct
DVQLQESGPGLVKPSQSLSLTCSVTGYSITSAYYWNWIRQFPGNKLECMGYISYDGSNYYNPSLKNRISITRDTSKNQFFLSLNSVTTEDTATYFCVRGGDYDDGGFAYWGQGTLVTVSA

SEQ ID NO: 81 - protein, 120 aa, synthetic construct
DVQLQESGPGLVKPSQSLSLTCSVTGYSITSGYYWNWIRQFPGNKLECMGYISYDGSNYYNPSLKNRISITRDTSKNQFFLSLNSVTTEDTATYFCVRGGDYDDGGFAYWGQGTLVTVSA

SEQ ID NO: 82 - protein, 121 aa, synthetic construct
EVQMVESGGDLVKPGDSLKLSCAASGFTFRSYGMSWVRQTPDKRLEWVATISSGDSYTYYPDSVKGRFTISRDNAKNTLYLQMSSLKSEDTALYYCARQIYYDYAYYFDFWGQGTTLTVSS

SEQ ID NO: 83 - protein, 111 aa, synthetic construct
DIVLTQSPASLAVSLGQRATISCRASESVSFRTSHLMHWYQQKPGQPPKLLIYGASNLESGVPARFSGSGSETDFTLNIHPVEEEDAAAYFCQQSIEDPPTFGGGTKLEIK

SEQ ID NO: 84 - protein, 120 aa, synthetic construct
DVQLQESGPGLVKPSQSLSLTCSVTGYSITSGYYWNWIRQFPGNKLECMGYITYDGSNNYNPSLKDRISITRDTSKNQFFLKLNSVTTEDTATYYCARGGDYDDGGFAYWGHGTLVTVSA

SEQ ID NO: 85 - protein, 107 aa, synthetic construct
DIQMTQSPVSLSASVGETVTITCRASGNIHNYLAWYQQKQGKSPQLLVYNAKSLVDGVPSRFSGSGSGTQYSLKINSLQPEDFGSYYCQHFWIIPYTFGGGTKLEIK

SEQ ID NO: 86 - protein, 15 aa, synthetic construct
KASQSIDYDAIGYLN

SEQ ID NO: 87 - protein, 121 aa, synthetic construct
EVQLVESGGGLVKPGGSLRLSCAASGFTFSSYGMSWVRQAPGKGLEWVSTISSGDSYTYYPDSVKGRFTISRDNAKNSLYLQMNSLRAEDTAVYYCARQIYYDYAYYFDFWGQGTTVTVSS

SEQ ID NO: 88 - protein, 121 aa, synthetic construct; identical to SEQ ID NO: 87

SEQ ID NO: 89 - protein, 121 aa, synthetic construct; identical to SEQ ID NO: 87

SEQ ID NO: 90 - protein, 121 aa, synthetic construct; identical to SEQ ID NO: 87

SEQ ID NO: 91 - protein, 121 aa, synthetic construct; identical to SEQ ID NO: 87

SEQ ID NO: 92 - protein, 121 aa, synthetic construct; identical to SEQ ID NO: 87

SEQ ID NO: 93 - protein, 121 aa, synthetic construct; identical to SEQ ID NO: 87

SEQ ID NO: 94 - protein, 121 aa, synthetic construct; identical to SEQ ID NO: 87

SEQ ID NO: 95 - protein, 121 aa, synthetic construct
EVQLVESGGGLVKPGGSLRLSCAASGFTFRSYGMSWVRQAPGKRLEWVSTISSGDSYTYYPDSVKGRFTISRDNAKNSLYLQMNSLRAEDTAVYYCARQIYYDYAYYFDFWGQGTTVTVSS

SEQ ID NO: 96 - protein, 121 aa, synthetic construct; identical to SEQ ID NO: 95

SEQ ID NO: 97 - protein, 121 aa, synthetic construct; identical to SEQ ID NO: 95

SEQ ID NO: 98 - protein, 121 aa, synthetic construct; identical to SEQ ID NO: 95

SEQ ID NO: 99 - protein, 121 aa, synthetic construct; identical to SEQ ID NO: 95

SEQ ID NO: 100 - protein, 121 aa, synthetic construct; identical to SEQ ID NO: 95

SEQ ID NO: 101 - protein, 121 aa, synthetic construct; identical to SEQ ID NO: 95

SEQ ID NO: 102 - protein, 121 aa, synthetic construct; identical to SEQ ID NO: 95

SEQ ID NO: 103 - protein, 121 aa, synthetic construct
EVQLVESGGGLVKPGGSLRLSCAASGFTFRSYGMSWVRQAPGKRLEWVSTISSGDSYTYYPDSVKGRFTISRDNAKNSLYLQMNSLKAEDTAVYYCARQIYYDYAYYFDFWGQGTTVTVSS

SEQ ID NO: 104 - protein, 121 aa, synthetic construct; identical to SEQ ID NO: 103

SEQ ID NO: 105 - protein, 121 aa, synthetic construct; identical to SEQ ID NO: 103

SEQ ID NO: 106 - protein, 121 aa, synthetic construct; identical to SEQ ID NO: 103

SEQ ID NO: 107 - protein, 121 aa, synthetic construct; identical to SEQ ID NO: 103

SEQ ID NO: 108 - protein, 121 aa, synthetic construct; identical to SEQ ID NO: 103

SEQ ID NO: 109 - protein, 121 aa, synthetic construct; identical to SEQ ID NO: 103

SEQ ID NO: 110 - protein, 121 aa, synthetic construct; identical to SEQ ID NO: 103

SEQ ID NO: 111 - protein, 120 aa, synthetic construct
QVQLQESGPGLVKPSETLSLTCTVSGGSISNYGVHWIRQPPGKGLEWIGVIWSGESTDYDAAFISRVTISVDTSKNQFSLKLSSVTAADTAVYYCARRRSHYYGYVMDYWGQGTTVTVSS

SEQ ID NO: 112 - protein, 120 aa, synthetic construct
QVQLQESGPGLVKPSETLSLTCTVSGGSISNYGVHWIRQPPGKGLEWIGVIWSGESTDYDAAFISRVTISKDNSKNQFSLKLSSVTAADTAVYYCARRRSHYYGYVMDYWGQGTTVTVSS

SEQ ID NO: 113 - protein, 120 aa, synthetic construct
QVQLQESGPGLVKPSETLSLTCTVSGGSITNYGVHWIRQPPGKGLEWIGVIWSGESTDYDAAFISRVTISKDNSKNQVSLKLSSVTAADTAVYYCARRRSHYYGYVMDYWGQGTTVTVSS

SEQ ID NO: 114 - protein, 120 aa, synthetic construct
QVQLQQSGPGLVKPSETLSLTCTVSGGSLTNYGVHWIRQPPGKGLEWIGVIWSGESTDYDAAFISRVTISKDNSKNQVSLKLSSVTAADTAVYYCARRRSHYYGYVMDYWGQGTTVTVSS

SEQ ID NO: 115 - protein, 120 aa, synthetic construct; identical to SEQ ID NO: 111

SEQ ID NO: 116 - protein, 120 aa, synthetic construct; identical to SEQ ID NO: 112

SEQ ID NO: 117 - protein, 120 aa, synthetic construct; identical to SEQ ID NO: 113

SEQ ID NO: 118 - protein, 120 aa, synthetic construct; identical to SEQ ID NO: 114

SEQ ID NO: 119 - protein, 120 aa, synthetic construct; identical to SEQ ID NO: 111

SEQ ID NO: 120 - protein, 120 aa, synthetic construct; identical to SEQ ID NO: 112

SEQ ID NO: 121 - protein, 120 aa, synthetic construct; identical to SEQ ID NO: 113

SEQ ID NO: 122 - protein, 120 aa, synthetic construct; identical to SEQ ID NO: 114

SEQ ID NO: 123 - protein, 120 aa, synthetic construct; identical to SEQ ID NO: 111

SEQ ID NO: 124 - protein, 120 aa, synthetic construct; identical to SEQ ID NO: 112

SEQ ID NO: 125 - protein, 120 aa, synthetic construct; identical to SEQ ID NO: 113

SEQ ID NO: 126 - protein, 120 aa, synthetic construct; identical to SEQ ID NO: 114

SEQ ID NO: 127 - protein, 120 aa, synthetic construct; identical to SEQ ID NO: 111

SEQ ID NO: 128 - protein, 120 aa, synthetic construct; identical to SEQ ID NO: 112

SEQ ID NO: 129 - protein, 120 aa, synthetic construct; identical to SEQ ID NO: 113

SEQ ID NO: 130 - protein, 120 aa, synthetic construct; identical to SEQ ID NO: 114

SEQ ID NO: 131 - protein, 120 aa, synthetic construct; identical to SEQ ID NO: 111

SEQ ID NO: 132 - protein, 120 aa, synthetic construct; identical to SEQ ID NO: 112

SEQ ID NO: 133 - protein, 120 aa, synthetic construct; identical to SEQ ID NO: 113

SEQ ID NO: 134 - protein, 120 aa, synthetic construct; identical to SEQ ID NO: 114

SEQ ID NO: 135 - protein, 111 aa, synthetic construct
DIVLTQSPASLAVSPGQRATITCRASESVSFRTSHLMHWYQQKPGQPPKLLIYGASNLESGVPARFSGSGSGTDFTLTINPVEANDTANYYCQQSIEDPPTFGGGTKVEIK

SEQ ID NO: 136 - protein, 111 aa, synthetic construct
DIVLTQSPASLAVSPGQRATITCRASESVSFRTSHLMHWYQQKPGQPPKLLIYGASNLESGVPARFSGSGSETDFTLTINPVEAEDTANYYCQQSIEDPPTFGGGTKVEIK

SEQ ID NO: 137 - protein, 111 aa, synthetic construct
DIVLTQSPASLAVSPGQRATITCRASESVSFRTSHLMHWYQQKPGQPPKLLIYGASNLESGVPARFSGSGSETDFTLTINPVEAEDTANYFCQQSIEDPPTFGGGTKVEIK

SEQ ID NO: 138 - protein, 111 aa, synthetic construct
DIVMTQSPDSLAVSLGERATINCRASESVSFRTSHLMHWYQQKPGQPPKLLIYGASNLESGVPDRFSGSGSGTDFTLTISSLQAEDVAVYYCQQSIEDPPTFGGGTKVEIK

SEQ ID NO: 139 - protein, 111 aa, synthetic construct
DIVLTQSPDSLAVSLGERATINCRASESVSFRTSHLMHWYQQKPGQPPKLLIYGASNLESGVPDRFSGSGSGTDFTLTISSLQAEDVAVYFCQQSIEDPPTFGGGTKVEIK

SEQ ID NO: 140 - protein, 111 aa, synthetic construct
DIVLTQSPDSLAVSLGERATINCRASESVSFRTSHLMHWYQQKPGQPPKLLIYGASNLESGVPDRFSGSGSETDFTLTISPLQAEDVAVYFCQQSIEDPPTFGGGTKVEIK

SEQ ID NO: 141 - protein, 111 aa, synthetic construct
EIVLTQSPATLSLSPGERATLSCRASESVSFRTSHLMHWYQQKPGQAPRLLIYGASNLESGIPARFSGSGSGTDFTLTISRLEPEDFAVYYCQQSIEDPPTFGGGTKVEIK

SEQ ID NO: 142 - protein, 111 aa, synthetic construct
EIVLTQSPATLSLSPGERATLSCRASESVSFRTSHLMHWYQQKPGQAPRLLIYGASNLESGIPARFSGSGSETDFTLTISRLEPEDFAVYFCQQSIEDPPTFGGGTKVEIK

SEQ ID NO: 143 - protein, 111 aa, synthetic construct; identical to SEQ ID NO: 135

SEQ ID NO: 144 - protein, 111 aa, synthetic construct; identical to SEQ ID NO: 136

SEQ ID NO: 145 - protein, 111 aa, synthetic construct; identical to SEQ ID NO: 137

SEQ ID NO: 146 - protein, 111 aa, synthetic construct; identical to SEQ ID NO: 138

SEQ ID NO: 147 - protein, 111 aa, synthetic construct; identical to SEQ ID NO: 139

SEQ ID NO: 148 - protein, 111 aa, synthetic construct; identical to SEQ ID NO: 140

SEQ ID NO: 149 - protein, 111 aa, synthetic construct; identical to SEQ ID NO: 141

SEQ ID NO: 150 - protein, 111 aa, synthetic construct; identical to SEQ ID NO: 142

SEQ ID NO: 151 - protein, 111 aa, synthetic construct; identical to SEQ ID NO: 135

SEQ ID NO: 152 - protein, 111 aa, synthetic construct; identical to SEQ ID NO: 136

SEQ ID NO: 153 - protein, 111 aa, synthetic construct; identical to SEQ ID NO: 137

SEQ ID NO: 154 - protein, 111 aa, synthetic construct; identical to SEQ ID NO: 138

SEQ ID NO: 155 - protein, 111 aa, synthetic construct; identical to SEQ ID NO: 139

SEQ ID NO: 156 - protein, 111 aa, synthetic construct; identical to SEQ ID NO: 140

SEQ ID NO: 157 - protein, 111 aa, synthetic construct; identical to SEQ ID NO: 141

SEQ ID NO: 158 - protein, 111 aa, synthetic construct; identical to SEQ ID NO: 142

SEQ ID NO: 159 - protein, 111 aa, synthetic construct
DIVLTQSPASLAVSPGQRATITCKASQSIDYDAIGYLNWYQQKPGQPPKLLIYAASNLESGVPARFSGSGSGTDFTLTINPVEANDTANYYCQQSNEDPPTFGQGTKLEIK

SEQ ID NO: 160 - protein, 111 aa, synthetic construct; identical to SEQ ID NO: 159

SEQ ID NO: 161 - protein, 111 aa, synthetic construct; identical to SEQ ID NO: 159

SEQ ID NO: 162 - protein, 111 aa, synthetic construct; identical to SEQ ID NO: 159

SEQ ID NO: 163 - protein, 111 aa, synthetic construct
DIVLTQSPASLAVSPGQRATITCKASQSIDYDAIGYLNWYQHKPGQPPKLLIYAASNLESGVPARFSGSGSGTDFTLTINPVEANDTANYYCQQSNEDPPTFGQGTKLEIK

SEQ ID NO: 164 - protein, 111 aa, synthetic construct; identical to SEQ ID NO: 163

SEQ ID NO: 165 - protein, 111 aa, synthetic construct; identical to SEQ ID NO: 163

SEQ ID NO: 166 - protein, 111 aa, synthetic construct; identical to SEQ ID NO: 163

SEQ ID NO: 167 - protein, 111 aa, synthetic construct
EIVLTQSPATLSLSPGERATLSCKASQSIDYDAIGYLNWYQQKPGQAPRLLIYAASNLESGIPARFSGSGSGTDFTLTISSLEPEDFAVYYCQQSNEDPPTFGQGTKLEIK

SEQ ID NO: 168 - protein, 111 aa, synthetic construct; identical to SEQ ID NO: 167

SEQ ID NO: 169 - protein, 111 aa, synthetic construct; identical to SEQ ID NO: 167

SEQ ID NO: 170 - protein, 111 aa, synthetic construct; identical to SEQ ID NO: 167

SEQ ID NO: 171 - protein, 111 aa, synthetic construct
EIVLTQSPATLSLSPGERATLSCKASQSIDYDAIGYLNWYQHKPGQAPRLLIYAASNLESGIPARFSGSGSGTDFTLTISSLEPEDFAVYYCQQSNEDPPTFGQGTKLEIK

SEQ ID NO: 172 - protein, 111 aa, synthetic construct; identical to SEQ ID NO: 171

SEQ ID NO: 173 - protein, 111 aa, synthetic construct; identical to SEQ ID NO: 171

SEQ ID NO: 174 - protein, 111 aa, synthetic construct; identical to SEQ ID NO: 171

SEQ ID NO: 175 - protein, 111 aa, synthetic construct
DIVMTQSPDSLAVSLGERATINCKASQSIDYDAIGYLNWYQQKPGQPPKLLIYAASNLESGVPDRFSGSGSGTDFTLTISSLQAEDVAVYYCQQSNEDPPTFGQGTKLEIK

SEQ ID NO: 176 - protein, 111 aa, synthetic construct; identical to SEQ ID NO: 175

SEQ ID NO: 177 - protein, 111 aa, synthetic construct; identical to SEQ ID NO: 175

SEQ ID NO: 178 - protein, 111 aa, synthetic construct; identical to SEQ ID NO: 175

SEQ ID NO: 179 - protein, 111 aa, synthetic construct
DIQMTQSPSSLSASVGDRVTITCKASQSIDYDAIGYLNWYQQKPGKAPKLLIYAASNLESGVPSRFSGSGSGTDFTLTISSLQPEDFATYYCQQSNEDPPTFGQGTKLEIK

SEQ ID NO: 180 - protein, 111 aa, synthetic construct; identical to SEQ ID NO: 179

SEQ ID NO: 181 - protein, 111 aa, synthetic construct; identical to SEQ ID NO: 179

SEQ ID NO: 182 - protein, 111 aa, synthetic construct; identical to SEQ ID NO: 179

SEQ ID NO: 183 - protein, 451 aa, synthetic construct
EVQLVESGGGLVKPGGSLRLSCAASGFTFSSYGMSWVRQAPGKGLEWVSTISSGDSYTYYPDSVKGRFTISRDNAKNSLYLQMNSLRAEDTAVYYCARQIYYDYAYYFDFWGQGTTVTVSSASTKGPSVFPLAPSSKSTSGGTAALGCLVKDYFPEPVTVSWNSGALTSGVHTFPAVLQSSGLYSLSSVVTVPSSSLGTQTYICNVNHKPSNTKVDKKVEPKSCDKTHTCPPCPAPELLGGPSVFLFPPKPKDTLMISRTPEVTCVVVDVSHEDPEVKFNWYVDGVEVHNAKTKPREEQYNSTYRVVSVLTVLHQDWLNGKEYKCKVSNKALPAPIEKTISKAKGQPREPQVYTLPPSRDELTKNQVSLTCLVKGFYPSDIAVEWESNGQPENNYKTTPPVLDSDGSFFLYSKLTVDKSRWQQGNVFSCSVMHEALHNHYTQKSLSLSPGK

SEQ ID NO: 184 - protein, 451 aa, synthetic construct
EVQLVESGGGLVKPGGSLRLSCAASGFTFRSYGMSWVRQAPGKRLEWVSTISSGDSYTYYPDSVKGRFTISRDNAKNSLYLQMNSLKAEDTAVYYCARQIYYDYAYYFDFWGQGTTVTVSSASTKGPSVFPLAPSSKSTSGGTAALGCLVKDYFPEPVTVSWNSGALTSGVHTFPAVLQSSGLYSLSSVVTVPSSSLGTQTYICNVNHKPSNTKVDKKVEPKSCDKTHTCPPCPAPELLGGPSVFLFPPKPKDTLMISRTPEVTCVVVDVSHEDPEVKFNWYVDGVEVHNAKTKPREEQYNSTYRVVSVLTVLHQDWLNGKEYKCKVSNKALPAPIEKTISKAKGQPREPQVYTLPPSRDELTKNQVSLTCLVKGFYPSDIAVEWESNGQPENNYKTTPPVLDSDGSFFLYSKLTVDKSRWQQGNVFSCSVMHEALHNHYTQKSLSLSPGK

SEQ ID NO: 185 - protein, 450 aa, synthetic construct
QVQLQQSGPGLVKPSETLSLTCTVSGGSLTNYGVHWIRQPPGKGLEWIGVIWSGESTDYDAAFISRVTISKDNSKNQVSLKLSSVTAADTAVYYCARRRSHYYGYVMDYWGQGTTVTVSSASTKGPSVFPLAPSSKSTSGGTAALGCLVKDYFPEPVTVSWNSGALTSGVHTFPAVLQSSGLYSLSSVVTVPSSSLGTQTYICNVNHKPSNTKVDKKVEPKSCDKTHTCPPCPAPELLGGPSVFLFPPKPKDTLMISRTPEVTCVVVDVSHEDPEVKFNWYVDGVEVHNAKTKPREEQYNSTYRVVSVLTVLHQDWLNGKEYKCKVSNKALPAPIEKTISKAKGQPREPQVYTLPPSRDELTKNQVSLTCLVKGFYPSDIAVEWESNGQPENNYKTTPPVLDSDGSFFLYSKLTVDKSRWQQGNVFSCSVMHEALHNHYTQKSLSLSPGK

SEQ ID NO: 186 - protein, 218 aa, synthetic construct
DIVLTQSPASLAVSPGQRATITCRASESVSFRTSHLMHWYQQKPGQPPKLLIYGASNLESGVPARFSGSGSETDFTLTINPVEAEDTANYFCQQSIEDPPTFGGGTKVEIKRTVAAPSVFIFPPSDEQLKSGTASVVCLLNNFYPREAKVQWKVDNALQSGNSQESVTEQDSKDSTYSLSSTLTLSKADYEKHKVYACEVTHQGLSSPVTKSFNRGEC

SEQ ID NO: 187 - protein, 218 aa, synthetic construct
DIVMTQSPDSLAVSLGERATINCRASESVSFRTSHLMHWYQQKPGQPPKLLIYGASNLESGVPDRFSGSGSGTDFTLTISSLQAEDVAVYYCQQSIEDPPTFGGGTKVEIKRTVAAPSVFIFPPSDEQLKSGTASVVCLLNNFYPREAKVQWKVDNALQSGNSQESVTEQDSKDSTYSLSSTLTLSKADYEKHKVYACEVTHQGLSSPVTKSFNRGEC

SEQ ID NO: 188 - protein, 218 aa, synthetic construct
DIVLTQSPASLAVSPGQRATITCKASQSIDYDAIGYLNWYQQKPGQPPKLLIYAASNLESGVPARFSGSGSGTDFTLTINPVEANDTANYYCQQSNEDPPTFGQGTKLEIKRTVAAPSVFIFPPSDEQLKSGTASVVCLLNNFYPREAKVQWKVDNALQSGNSQESVTEQDSKDSTYSLSSTLTLSKADYEKHKVYACEVTHQGLSSPVTKSFNRGEC

SEQ ID NO: 189 - protein, 426 aa, synthetic construct
MDMRVPAQLLGLLLLWFPGSRCPKSCDKTHTCPPCPAPELLGGPSVFLFPPKPKDTLMISRTPEVTCVVVDVSHEDPEVKFNWYVDGVEVHNAKTKPREEQYNSTYRVVSVLTVLHQDWLNGKEYKCKVSNKALPAPIEKTISKAKGQPREPQVYTLPPSRDELTKNQVSLTCLVKGFYPSDIAVEWESNGQPENNYKTTPPVLDSDGSFFLYSKLTVDKSRWQQGNVFSCSVMHEALHNHYTQKSLSLSPGKIEGRNFMYSKTVKRLSKLREYQQYHPSLTCVMEGKDIEDWSCCPTPWTSFQSSCYFISTGMQSWTKSQKNCSVMGADLVVINTREEQDFIIQNLKRNSSYFLGLSDPGGRRHWQWVDQTPYNENVTFWHSGEPNNLDERCAIINFRSSEEWGWNDIHCHVPQKSICKMKKIYI

SEQ ID NO: 190 - protein, 196 aa, synthetic construct
MDMRVPAQLLGLLLLWFPGSRCHHHHHHNFMYSKTVKRLSKLQEYQQYYPSLTCVMEGKDMEDWSCCPTPWTSFQSSCYFISTVMQSWTKSQNNCSVMGADLVVINTKEEQDFITQNLKINSAYFLGLSDPKGWRHWQWVDQTPYNKNVTFWHSGEPNSPDERCAIINFRSEEWGWNDVHCHVPQKSICKMKKIYI

SEQ ID NO: 191 - protein, 451 aa, synthetic construct
EVQLVESGGGLVKPGGSLRLSCAASGFTFSSYGMSWVRQAPGKGLEWVSTISSGDSYTYYPDSVKGRFTISRDNAKNSLYLQMNSLRAEDTAVYYCARQIYYDYAYYFDFWGQGTTVTVSSASTKGPSVFPLAPSSKSTSGGTAALGCLVKDYFPEPVTVSWNSGALTSGVHTFPAVLQSSGLYSLSSVVTVPSSSLGTQTYICNVNHKPSNTKVDKKVEPKSCDKTHTCPPCPAPELLGGPDVFLFPPKPKDTLMISRTPEVTCVVVDVSHEDPEVKFNWYVDGVEVHNAKTKPREEQYNSTYRVVSVLTVLHQDWLNGKEYKCKVSNKALPAPEEKTISKAKGQPREPQVYTLPPSRDELTKNQVSLTCLVKGFYPSDIAVEWESNGQPENNYKTTPPVLDSDGSFFLYSKLTVDKSRWQQGNVFSCSVMHEALHNHYTQKSLSLSPGK

SEQ ID NO: 192 - protein, 451 aa, synthetic construct
EVQLVESGGGLVKPGGSLRLSCAASGFTFSSYGMSWVRQAPGKGLEWVSTISSGDSYTYYPDSVKGRFTISRDNAKNSLYLQMNSLRAEDTAVYYCARQIYYDYAYYFDFWGQGTTVTVSSASTKGPSVFPLAPSSKSTSGGTAALGCLVKDYFPEPVTVSWNSGALTSGVHTFPAVLQSSGLYSLSSVVTVPSSSLGTQTYICNVNHKPSNTKVDKKVEPKSCDKTHTCPPCPAPELLAGPDVFLFPPKPKDTLMISRTPEVTCVVVDVSHEDPEVKFNWYVDGVEVHNAKTKPREEQYNSTYRVVSVLTVLHQDWLNGKEYKCKVSNKALPAPEEKTISKAKGQPREPQVYTLPPSRDELTKNQVSLTCLVKGFYPSDIAVEWESNGQPENNYKTTPPVLDSDGSFFLYSKLTVDKSRWQQGNVFSCSVMHEALHNHYTQKSLSLSPGK

SEQ ID NO: 193 - protein, 451 aa, synthetic construct
EVQLVESGGGLVKPGGSLRLSCAASGFTFSSYGMSWVRQAPGKGLEWVSTISSGDSYTYYPDSVKGRFTISRDNAKNSLYLQMNSLRAEDTAVYYCARQIYYDYAYYFDFWGQGTTVTVSSASTKGPSVFPLAPSSKSTSGGTAALGCLVKDYFPEPVTVSWNSGALTSGVHTFPAVLQSSGLYSLSSVVTVPSSSLGTQTYICNVNHKPSNTKVDKKVEPKSCDKTHTCPPCPAPELLAGPSVFLFPPKPKDTLMISRTPEVTCVVVDVSHEDPEVKFNWYVDGVEVHNAKTKPREEQYNSTYRVVSVLTVLHQDWLNGKEYKCKVSNKALPAPEEKTISKAKGQPREPQVYTLPPSRDELTKNQVSLTCLVKGFYPSDIAVEWESNGQPENNYKTTPPVLDSDGSFFLYSKLTVDKSRWQQGNVFSCSVMHEALHNHYTQKSLSLSPGK

SEQ ID NO: 194 - protein, 451 aa, synthetic construct
EVQLVESGGGLVKPGGSLRLSCAASGFTFRSYGMSWVRQAPGKRLEWVSTISSGDSYTYYPDSVKGRFTISRDNAKNSLYLQMNSLKAEDTAVYYCARQIYYDYAYYFDFWGQGTTVTVSSASTKGPSVFPLAPSSKSTSGGTAALGCLVKDYFPEPVTVSWNSGALTSGVHTFPAVLQSSGLYSLSSVVTVPSSSLGTQTYICNVNHKPSNTKVDKKVEPKSCDKTHTCPPCPAPELLGGPDVFLFPPKPKDTLMISRTPEVTCVVVDVSHEDPEVKFNWYVDGVEVHNAKTKPREEQYNSTYRVVSVLTVLHQDWLNGKEYKCKVSNKALPAPEEKTISKAKGQPREPQVYTLPPSRDELTKNQVSLTCLVKGFYPSDIAVEWESNGQPENNYKTTPPVLDSDGSFFLYSKLTVDKSRWQQGNVFSCSVMHEALHNHYTQKSLSLSPGK

SEQ ID NO: 195 - protein, 451 aa, synthetic construct
EVQLVESGGGLVKPGGSLRLSCAASGFTFRSYGMSWVRQAPGKRLEWVSTISSGDSYTYYPDSVKGRFTISRDNAKNSLYLQMNSLKAEDTAVYYCARQIYYDYAYYFDFWGQGTTVTVSSASTKGPSVFPLAPSSKSTSGGTAALGCLVKDYFPEPVTVSWNSGALTSGVHTFPAVLQSSGLYSLSSVVTVPSSSLGTQTYICNVNHKPSNTKVDKKVEPKSCDKTHTCPPCPAPELLAGPDVFLFPPKPKDTLMISRTPEVTCVVVDVSHEDPEVKFNWYVDGVEVHNAKTKPREEQYNSTYRVVSVLTVLHQDWLNGKEYKCKVSNKALPAPEEKTISKAKGQPREPQVYTLPPSRDELTKNQVSLTCLVKGFYPSDIAVEWESNGQPENNYKTTPPVLDSDGSFFLYSKLTVDKSRWQQGNVFSCSVMHEALHNHYTQKSLSLSPGK

SEQ ID NO: 196 - protein, 451 aa, synthetic construct
EVQLVESGGGLVKPGGSLRLSCAASGFTFRSYGMSWVRQAPGKRLEWVSTISSGDSYTYYPDSVKGRFTISRDNAKNSLYLQMNSLKAEDTAVYYCARQIYYDYAYYFDFWGQGTTVTVSSASTKGPSVFPLAPSSKSTSGGTAALGCLVKDYFPEPVTVSWNSGALTSGVHTFPAVLQSSGLYSLSSVVTVPSSSLGTQTYICNVNHKPSNTKVDKKVEPKSCDKTHTCPPCPAPELLAGPSVFLFPPKPKDTLMISRTPEVTCVVVDVSHEDPEVKFNWYVDGVEVHNAKTKPREEQYNSTYRVVSVLTVLHQDWLNGKEYKCKVSNKALPAPEEKTISKAKGQPREPQVYTLPPSRDELTKNQVSLTCLVKGFYPSDIAVEWESNGQPENNYKTTPPVLDSDGSFFLYSKLTVDKSRWQQGNVFSCSVMHEALHNHYTQKSLSLSPGK